European Patent Specification EP 3 332 006 B1, published October 11, 2023. Title: NOVEL ANTI-PD-L1 ANTIBODIES. Applicant: WuXi Biologics (Shanghai) Co. Ltd. Open Monoclonal Technology, Inc. The sequence listing filed with the application follows.

SEQUENCE LISTING (56 sequences)

SEQ ID NO: 1 - protein, 7 aa, Homo sapiens
IRTYYWG

SEQ ID NO: 2 - DNA, 21 bp, Homo sapiens
attagaacttactactggggc

SEQ ID NO: 3 - protein, 16 aa, Homo sapiens
YIYYSGSTRYNPSLKS

SEQ ID NO: 4 - DNA, 48 bp, Homo sapiens
tatatctattatagtgggagcacccgctacaacccgtccctcaagagt

SEQ ID NO: 5 - protein, 7 aa, Homo sapiens
LSYFFDY

SEQ ID NO: 6 - DNA, 21 bp, Homo sapiens
cttagctacttctttgactac

SEQ ID NO: 7 - protein, 11 aa, Homo sapiens
SGDKLGDKYAC

SEQ ID NO: 8 - DNA, 33 bp, Homo sapiens
tctggagataaattgggggataaatatgcttgc

SEQ ID NO: 9 - protein, 7 aa, Homo sapiens
QDTKRPS

SEQ ID NO: 10 - DNA, 21 bp, Homo sapiens
caagataccaagcggccctca

SEQ ID NO: 11 - protein, 9 aa, Homo sapiens
QAWDSGTVI

SEQ ID NO: 12 - DNA, 27 bp, Homo sapiens
caggcgtgggacagcggcactgtgata

SEQ ID NO: 13 - protein, 5 aa, Homo sapiens
SYAMS

SEQ ID NO: 14 - DNA, 15 bp, Homo sapiens
agctatgccatgagt

SEQ ID NO: 15 - protein, 17 aa, Homo sapiens
GISGSGGFTYYADSVKG

SEQ ID NO: 16 - DNA, 51 bp, Homo sapiens
ggtattagtggtagtggtggtttcacttactacgcagactccgtgaagggc

SEQ ID NO: 17 - protein, 12 aa, Homo sapiens
PPRGYNYGPFDY

SEQ ID NO: 18 - DNA, 36 bp, Homo sapiens
cctcctcgtggatacaactatggcccttttgactac

SEQ ID NO: 19 - protein, 11 aa, Homo sapiens
GGNNIGSKSVH

SEQ ID NO: 20 - DNA, 33 bp, Homo sapiens
gggggaaacaacattggaagtaaaagtgtacac

SEQ ID NO: 21 - protein, 7 aa, Homo sapiens
DDSDRPS

SEQ ID NO: 22 - DNA, 21 bp, Homo sapiens
gatgatagcgaccggccctca

SEQ ID NO: 23 - protein, 11 aa, Homo sapiens
QVWDSSSDHVV

SEQ ID NO: 24 - DNA, 33 bp, Homo sapiens
caggtgtgggatagtagtagtgatcacgtggta

SEQ ID NO: 25 - protein, 7 aa, Homo sapiens
SISNYWG

SEQ ID NO: 26 - DNA, 21 bp, Homo sapiens
agtattagtaactactggggc

SEQ ID NO: 27 - protein, 16 aa, Homo sapiens
SIYYSGSTNYNPPLKS

SEQ ID NO: 28 - DNA, 48 bp, Homo sapiens
agtatctattatagtgggagcacgaactacaatccgcccctcaagagt

SEQ ID NO: 29 - protein, 7 aa, Homo sapiens
LTYYFDY

SEQ ID NO: 30 - DNA, 21 bp, Homo sapiens
ctgacctactactttgattac

SEQ ID NO: 31 - protein, 11 aa, Homo sapiens
SGDKLGDKYAC

SEQ ID NO: 32 - DNA, 33 bp, Homo sapiens; identical to SEQ ID NO: 8

SEQ ID NO: 33 - protein, 7 aa, Homo sapiens
QDSKRPS

SEQ ID NO: 34 - DNA, 21 bp, Homo sapiens
caagatagcaagcggccctca

SEQ ID NO: 35 - protein, 9 aa, Homo sapiens
QTWDSSTVV

SEQ ID NO: 36 - DNA, 27 bp, Homo sapiens
cagacgtgggacagcagcactgtggta

SEQ ID NO: 37 - protein, 5 aa, Homo sapiens
SYAMS

SEQ ID NO: 38 - DNA, 15 bp, Homo sapiens
agctatgccatgagt

SEQ ID NO: 39 - protein, 17 aa, Homo sapiens
GFSGSGFITYYADSVKG

SEQ ID NO: 40 - DNA, 51 bp, Homo sapiens
ggttttagtggtagtggttttattacatactacgcagactccgtgaagggc

SEQ ID NO: 41 - protein, 12 aa, Homo sapiens
PPRGYNYGPFDY

SEQ ID NO: 42 - DNA, 36 bp, Artificial Sequence; identical to SEQ ID NO: 18
  Recombinant

SEQ ID NO: 43 - protein, 117 aa, Homo sapiens
QLQLQESGPGLVKPSESLSLTCTVSGGSISIRTYYWGWIRQPPGTGLEWMGYIYYSGSTRYNPSLKSRVTISVDTSKNQFSLKLSSVTAADTAVYYCARLSYFFDYWGQGTLVTVSS

SEQ ID NO: 44 - DNA, 351 bp, Homo sapiens
cagctgcaactgcaggagtcgggcccaggactggtgaagccttcggagtccctgtccctcacctgcactgtctctggtggctccatcagcattagaacttactactggggctggatccgccagcccccagggacggggctggagtggatggggtatatctattatagtgggagcacccgctacaacccgtccctcaagagtcgagtcaccatatccgtagacacgtccaagaaccagttctccctgaagctgagctctgtgaccgccgcagacacggctgtgtattactgtgcgagacttagctacttctttgactactggggccagggaaccctggtcaccgtctcctca

SEQ ID NO: 45 - protein, 106 aa, Homo sapiens
SYELTQPPSVSVSPGQTASITCSGDKLGDKYACWYQQKPGQSPVMVIYQDTKRPSGIPERFSGSNSGNTATLTISGTLAMDEADYYCQAWDSGTVIFGGGTKLTVL

SEQ ID NO: 46 - DNA, 318 bp, Homo sapiens
tcctatgaactgactcagccaccctcagtgtccgtgtccccaggacagacagccagcatcacctgctctggagataaattgggggataaatatgcttgctggtatcagcagaagccaggccagtcccctgtgatggtcatctatcaagataccaagcggccctcagggatccctgagcgattctctggctccaactctgggaacacagccactctgaccatcagcgggaccctggctatggatgaggctgactattattgtcaggcgtgggacagcggcactgtgatattcggcggagggaccaagctgaccgtccta

SEQ ID NO: 47 - protein, 121 aa, Homo sapiens
EVQLLESGGGLVQPGGSLRLSCAASGFTFSSYAMSWVRQAPGKGLEWVSGISGSGGFTYYADSVKGRFTISRDNSKNTLYLQMNSLRAEDTAVYYCAKPPRGYNYGPFDYWGQGTLVTVSS

SEQ ID NO: 48 - DNA, 363 bp, Homo sapiens
gaggtgcaactgttggagtctgggggaggcttggtacagcctggggggtccctgagactctcctgtgcagcctctggattcacctttagcagctatgccatgagttgggtccgccaggctccagggaaggggctggagtgggtctcaggtattagtggtagtggtggtttcacttactacgcagactccgtgaagggccggttcaccatctccagagacaattccaagaacacgctgtatctgcaaatgaacagcctgagagccgaggacacggccgtatattactgtgcgaaacctcctcgtggatacaactatggcccttttgactactggggccagggaaccctggtcaccgtctcctca

SEQ ID NO: 49 - protein, 108 aa, Homo sapiens
SYVLTQPPSVSVAPGQTARITCGGNNIGSKSVHWYQQKPGQAPVLVVYDDSDRPSGIPERFSGSNSGNTATLTISRVEAGDEADYYCQVWDSSSDHVVFGGGTKLTVL

SEQ ID NO: 50 - DNA, 324 bp, Homo sapiens
tcctatgtgctgactcagccaccctcggtgtcagtggccccaggacagacggccaggattacctgtgggggaaacaacattggaagtaaaagtgtacactggtaccagcagaagccaggccaggcccctgtgctggtcgtctatgatgatagcgaccggccctcagggatccctgagcgattctctggctccaactctgggaacacggccaccctgaccatcagcagggtcgaagccggggatgaggccgactattactgtcaggtgtgggatagtagtagtgatcacgtggtattcggcggagggaccaagctgaccgtccta

SEQ ID NO: 51 - protein, 117 aa, Homo sapiens
QLQLQESGPGLVKPSETLSLTCTVSGGSISSISNYWGWIRQPPGKGLEWIGSIYYSGSTNYNPPLKSRVTISVDTTKNQFSLKLSSVTAADTAVYYCARLTYYFDYWGQGMLVTVSS

SEQ ID NO: 52 - DNA, 351 bp, Homo sapiens
cagctgcagctgcaggagtcgggcccaggactggtgaagccttcggagaccctgtccctcacctgcactgtctctggtggctccatcagcagtattagtaactactggggctggatccgccagcccccagggaaggggctggagtggattgggagtatctattatagtgggagcacgaactacaatccgcccctcaagagtcgagtcaccatatccgtagacacgaccaagaaccagttctccctgaagctgagctctgtgaccgccgcagacacggctgtgtattactgtgcgagactgacctactactttgattactggggccagggaatgctggtcaccgtctcctca

SEQ ID NO: 53 - protein, 106 aa, Homo sapiens
SYDLTQPPSVSVSPGQTASITCSGDKLGDKYACWYQQKPGQSPLLVIQQDSKRPSGIPARFSGSNSGNTATLTISGTQAMDEADYFCQTWDSSTVVFGGGTKLTVL

SEQ ID NO: 54 - DNA, 318 bp, Homo sapiens
tcctatgacctgactcagccaccctcagtgtccgtctccccaggacagacagccagcatcacctgctctggagataaattgggggataaatatgcttgctggtatcagcagaagccaggccagtcccctttgctggtcatccagcaagatagcaagcggccctcagggatccctgcgcgattctctggctccaactctgggaacacagccactctgaccatcagcgggacccaggctatggatgaggctgactatttctgtcagacgtgggacagcagcactgtggtattcggcggagggaccaagctgaccgtccta

SEQ ID NO: 55 - protein, 121 aa, Homo sapiens
EVQLLESGGGLVQPGGSLRLSCAASGFTFSSYAMSWVRQAPGKGLEWVSGFSGSGFITYYADSVKGRFTISRDNSKNTLYLQMNSLRAEDTAVYYCAMPPRGYNYGPFDYWGQGTLVTVSS

SEQ ID NO: 56 - DNA, 363 bp, Homo sapiens
gaggtgcagttgttggagtctgggggaggcttggtacagcctggggggtccctgagactctcctgtgcagcctctggattcacctttagcagctatgccatgagttgggtccgccaggctccagggaaggggctggagtgggtctcaggttttagtggtagtggttttattacatactacgcagactccgtgaagggccggttcaccatctccagagacaattccaagaatacgctgtatctgcaaatgaacagcctgagagccgaggacacggccgtatattactgtgcgatgcctcctcgtggatacaactatggcccttttgactactggggccagggaaccctggtcaccgtctcctca